European Patent Specification EP 3 737 750 B1, published June 5, 2024. Title: ALKALINE PHOSPHATASE AGENTS FOR TREATMENT OF NEURODEVELOPMENTAL DISORDERS. Applicant: Synthetic Biologics, Inc. Kaleko, Michael Furlan Freguia, Christian Connelly, Sheila. The sequence listing filed with the application follows.

SEQUENCE LISTING (18 sequences)

SEQ ID NO: 1 - protein, 528 aa, Artificial Sequence
  Synthetic polymer
MQGPWVLLLLGLRLQLSLGVIPAEEENPAFWNRQAAEALDAAKKLQPIQKVAKNLILFLGDGLGVPTVTATRILKGQKNGKLGPETPLAMDRFPYLALSKTYNVDRQVPDSAATATAYLCGVKANFQTIGLSAAARFNQCNTTRGNEVISVMNRAKQAGKSVGVVTTTRVQHASPAGTYAHTVNRNWYSDADMPASARQEGCQDIATQLISNMDIDVILGGGRKYMFPMGTPDPEYPADASQNGIRLDGKNLVQEWLAKHQGAWYVWNRTELMQASLDQSVTHLMGLFEPGDTKYEIHRDPTLDPSLMEMTEAALRLLSRNPRGFYLFVEGGRIDHGHHEGVAYQALTEAVMFDDAIERAGQLTSEEDTLTLVTADHSHVFSFGGYTLRGSSIFGLAPSKAQDSKAYTSILYGNGPGYVFNSGVRPDVNESESGSPDYQQQAAVPLSSETHGGEDVAVFARGPQAHLVHGVQEQSFVAHVMAFAACLEPYTACDLAPPACTTDAAHPVAASLPLLAGTLLLLGASAAP

SEQ ID NO: 2 - protein, 533 aa, Artificial Sequence
  Synthetic polymer
MQGACVLLLLGLHLQLSLGLIPAEEENPAFWNRQAAQALDVAKKLQPIQTAAKNVILFLGDGMGVPTVTATRILKGQMNGKLGPETPLAMDQFPYVALSKTYNVDRQVPDSAGTATAYLCGVKGNYRTIGVSAAARYNQCNTTRGNEVTSVINRAKKAGKAVGVVTTTRVQHASPAGAYAHTVNRNWYSDADLPADAQKNGCQDIAAQLVYNMDIDVILGGGRMYMFPEGTPDPEYPDDASVNGVRKDKQNLVQEWQAKHQGAQYVWNRTALLQAADDSSVTHLMGLFEPADMKYNVQQDHTKDPTLAEMTEAALQVLSRNPRGFYLFVEGGRIDHGHHDGKAYMALTEAIMFDNAIAKANELTSELDTLILVTADHSHVFSFGGYTLRGTSIFGLAPGKALDSKSYTSILYGNGPGYALGGGSRPDVNGSTSEEPSYRQQAAVPLASETHGGEDVAVFARGPQAHLVHGVQEETFVAHIMAFAGCVEPYTDCNLPAPATATSIPDAAHLAASPPPLALLAGAMLLLLAPTLY

SEQ ID NO: 3 - protein, 530 aa, Artificial Sequence
  Synthetic polymer
MQWACVLLLLGLWLQLSLTFIPAEEEDPAFWNRQAAQALDVAKKLQPIQTAAKNVILFLGDGMGVPTVTATRILKGQMNGKLGPETPLAMDQFPYVALSKTYNVDRQVPDSAGTATAYLCGVKGNYKTIGVSAAARYNQCNTTSGNEVTSVMNRAKKAGKSVGVVTTSRVQHASPAGAYAHTVNRNWYSDADLPADAQTYGCQDIATQLVNNMDIDVILGGGRMYMFPEGTPDPEYPYDVNQTGVRKDKRNLVQEWQAKHQGAQYVWNRTELLQAANDPSVTHLMGLFEPADMKYNVQQDPTKDPTLEEMTEAALQVLSRNPQGFYLFVEGGRIDHGHHEGKAYMALTDTVMFDNAIAKANELTSELDTLILATADHSHVFSFGGYTLRGTSIFGLAPSKASDNKSYTSILYGNGPGYVLGGGLRPDVNDSISEDPSYRQQAAVPLSSESHGGEDVAVFARGPQAHLVHGVQEETFVAHVMAFAGCVEPYTDCNLPAPSGLSDAAHLAASPPSLALLAGAMLLLLAPALY

SEQ ID NO: 4 - protein, 503 aa, Artificial Sequence
  Synthetic polymer
MQGPWVLLLLGLRLQLSLGVIPAEEENPAFWNRQAAEALDAAKKLQPIQKVAKNLILFLGDGLGVPTVTATRILKGQKNGKLGPETPLAMDRFPYLALSKTYNVDRQVPDSAATATAYLCGVKANFQTIGLSAAARFNQCNTTRGNEVISVMNRAKQAGKSVGVVTTTRVQHASPAGTYAHTVNRNWYSDADMPASARQEGCQDIATQLISNMDIDVILGGGRKYMFPMGTPDPEYPADASQNGIRLDGKNLVQEWLAKHQGAWYVWNRTELMQASLDQSVTHLMGLFEPGDTKYEIHRDPTLDPSLMEMTEAALRLLSRNPRGFYLFVEGGRIDHGHHEGVAYQALTEAVMFDDAIERAGQLTSEEDTLTLVTADHSHVFSFGGYTLRGSSIFGLAPSKAQDSKAYTSILYGNGPGYVFNSGVRPDVNESESGSPDYQQQAAVPLSSETHGGEDVAVFARGPQAHLVHGVQEQSFVAHVMAFAACLEPYTACDLAPPAGTTD

SEQ ID NO: 5 - protein, 506 aa, Artificial Sequence
  Synthetic polymer
MQGACVLLLLGLHLQLSLGLIPAEEENPAFWNRQAAQALDVAKKLQPIQTAAKNVILFLGDGMGVPTVTATRILKGQMNGKLGPETPLAMDQFPYVALSKTYNVDRQVPDSAGTATAYLCGVKGNYRTIGVSAAARYNQCNTTRGNEVTSVINRAKKAGKAVGVVTTTRVQHASPAGAYAHTVNRNWYSDADLPADAQKNGCQDIAAQLVYNMDIDVILGGGRMYMFPEGTPDPEYPDDASVNGVRKDKQNLVQEWQAKHQGAQYVWNRTALLQAADDSSVTHLMGLFEPADMKYNVQQDHTKDPTLAEMTEAALQVLSRNPRGFYLFVEGGRIDHGHHDGKAYMALTEAIMFDNAIAKANELTSELDTLILVTADHSHVFSFGGYTLRGTSIFGLAPGKALDSKSYTSILYGNGPGYALGGGSRPDVNGSTSEEPSYRQQAAVPLASETHGGEDVAVFARGPQAHLVHGVQEETFVAHIMAFAGCVEPYTDCNLPAPATATSIPD

SEQ ID NO: 6 - protein, 503 aa, Artificial Sequence
  Synthetic polymer
MQWACVLLLLGLWLQLSLTFIPAEEEDPAFWNRQAAQALDVAKKLQPIQTAAKNVILFLGDGMGVPTVTATRILKGQMNGKLGPETPLAMDQFPYVALSKTYNVDRQVPDSAGTATAYLCGVKGNYKTIGVSAAARYNQCNTTSGNEVTSVMNRAKKAGKSVGVVTTSRVQHASPAGAYAHTVNRNWYSDADLPADAQTYGCQDIATQLVNNMDIDVILGGGRMYMFPEGTPDPEYPYDVNQTGVRKDKRNLVQEWQAKHQGAQYVWNRTELLQAANDPSVTHLMGLFEPADMKYNVQQDPTKDPTLEEMTEAALQVLSRNPQGFYLFVEGGRIDHGHHEGKAYMALTDTVMFDNAIAKANELTSELDTLILATADHSHVFSFGGYTLRGTSIFGLAPSKASDNKSYTSILYGNGPGYVLGGGLRPDVNDSISEDPSYRQQAAVPLSSESHGGEDVAVFARGPQAHLVHGVQEETFVAHVMAFAGCVEPYTDCNLPAPSGLSD

SEQ ID NO: 7 - protein, 508 aa, Artificial Sequence
  Synthetic polymer
MQWACVLLLLGLWLQLSLTFIPAEEEDPAFWNRQAAQALDVAKKLQPIQTAAKNVILFLGDGMGVPTVTATRILKGQMNGKLGPETPLAMDQFPYVALSKTYNVDRQVPDSAGTATAYLCGVKGNYKTIGVSAAARYNQCNTTSGNEVTSVMNRAKKAGKSVGVVTTSRVQHASPAGAYAHTVNRNWYSDADLPADAQTYGCQDIATQLVNNMDIDVILGGGRMYMFPEGTPDPEYPYDVNQTGVRKDKRNLVQEWQAKHQGAQYVWNRTELLQAANDPSVTHLMGLFEPADMKYNVQQDPTKDPTLEEMTEAALQVLSRNPQGFYLFVEGGRIDHGHHEGKAYMALTDTVMFDNAIAKANELTSELDTLILATADHSHVFSFGGYTLRGTSIFGLAPSKASDNKSYTSILYGNGPGYVLGGGLRPDVNDSISEDPSYRQQAAVPLSSESHGGEDVAVFARGPQAHLVHGVQEETFVAHVMAFAGCVEPYTDCNLPAPSGLSDAAHLA

SEQ ID NO: 8 - protein, 754 aa, Artificial Sequence
  Synthetic polymer
MQGACVLLLLGLHLQLSLGLIPAEEENPAFWNRQAAQALDVAKKLQPIQTAAKNVILFLGDGMGVPTVTATRILKGQMNGKLGPETPLAMDQFPYVALSKTYNVDRQVPDSAGTATAYLCGVKGNYRTIGVSAAARYNQCNTTRGNEVTSVINRAKKAGKAVGVVTTTRVQHASPAGAYAHTVNRNWYSDADLPADAQKNGCQDIAAQLVYNMDIDVILGGGRMYMFPEGTPDPEYPDDASVNGVRKDKQNLVQEWQAKHQGAQYVWNRTALLQAADDSSVTHLMGLFEPADMKYNVQQDHTKDPTLAEMTEAALQVLSRNPRGFYLFVEGGRIDHGHHDGKAYMALTEAIMFDNAIAKANELTSELDTLILVTADHSHVFSFGGYTLRGTSIFGLAPGKALDSKSYTSILYGNGPGYALGGGSRPDVNGSTSEEPSYRQQAAVPLASETHGGEDVAVFARGPQAHLVHGVQEETFVAHIMAFAGCVEPYTDCNLPAPATATSIPDGGSGGSGGGGSGGGGSEPKSCDKTHTCPPCPAPELLGGPSVFLFPPKPKDTLMISRTPEVTCVVVDVSHEDPQVKFNWYVDGVQVHNAKTKPREQQYNSTYRVVSVLTVLHQNWLDGKEYKCKVSNKALPAPIEKTISKAKGQPREPQVYTLPPSREEMTKNQVSLTCLVKGFYPSDIAVEWESNGQPENNYKTTPPVLDSDGSFFLYSKLTVDKSRWQQGNVFSCSVMHEALHNHYTQKSLSLSPGK

SEQ ID NO: 9 - protein, 751 aa, Artificial Sequence
  Synthetic polymer
MQWACVLLLLGLWLQLSLTFIPAEEEDPAFWNRQAAQALDVAKKLQPIQTAAKNVILFLGDGMGVPTVTATRILKGQMNGKLGPETPLAMDQFPYVALSKTYNVDRQVPDSAGTATAYLCGVKGNYKTIGVSAAARYNQCNTTSGNEVTSVMNRAKKAGKSVGVVTTSRVQHASPAGAYAHTVNRNWYSDADLPADAQTYGCQDIATQLVNNMDIDVILGGGRMYMFPEGTPDPEYPYDVNQTGVRKDKRNLVQEWQAKHQGAQYVWNRTELLQAANDPSVTHLMGLFEPADMKYNVQQDPTKDPTLEEMTEAALQVLSRNPQGFYLFVEGGRIDHGHHEGKAYMALTDTVMFDNAIAKANELTSELDTLILATADHSHVFSFGGYTLRGTSIFGLAPSKASDNKSYTSILYGNGPGYVLGGGLRPDVNDSISEDPSYRQQAAVPLSSESHGGEDVAVFARGPQAHLVHGVQEETFVAHVMAFAGCVEPYTDCNLPAPSGLSDGGSGGSGGGGSGGGGSEPKSCDKTHTCPPCPAPELLGGPSVFLFPPKPKDTLMISRTPEVTCVVVDVSHEDPQVKFNWYVDGVQVHNAKTKPREQQYNSTYRVVSVLTVLHQNWLDGKEYKCKVSNKALPAPIEKTISKAKGQPREPQVYTLPPSREEMTKNQVSLTCLVKGFYPSDIAVEWESNGQPENNYKTTPPVLDSDGSFFLYSKLTVDKSRWQQGNVFSCSVMHEALHNHYTQKSLSLSPGK

SEQ ID NO: 10 - protein, 539 aa, Artificial Sequence
  Synthetic polymer
MQWACVLLLLGLWLQLSLTFIPAEEEDPAFWNRQAAQALDVAKKLQPIQTAAKNVILFLGDGMGVPTVTATRILKGQMNGKLGPETPLAMDQFPYVALSKTYNVDRQVPDSAGTATAYLCGVKGNYKTIGVSAAARYNQCNTTSGNEVTSVMNRAKKAGKSVGVVTTSRVQHASPAGAYAHTVNRNWYSDADLPADAQTYGCQDIATQLVNNMDIDVILGGGRMYMFPEGTPDPEYPYDVNQTGVRKDKRNLVQEWQAKHQGAQYVWNRTELLQAANDPSVTHLMGLFEPADMKYNVQQDPTKDPTLEEMTEAALQVLSRNPQGFYLFVEGGRIDHGHHEGKAYMALTDTVMFDNAIAKANELTSELDTLILATADHSHVFSFGGYTLRGTSIFGLAPSKASDNKSYTSILYGNGPGYVLGGGLRPDVNDSISEDPSYRQQAAVPLSSESHGGEDVAVFARGPQAHLVHGVQEETFVAHVMAFAGCVEPYTDCNLEVLFQGPAPPAGTTDAAHPGRSVVPALLPLRAGTLLLLETATAP

SEQ ID NO: 11 - protein, 534 aa, Artificial Sequence
  Synthetic polymer
MQWACVLLLLGLWLQLSLTFIPAEEEDPAFWNRQAAQALDVAKKLQPIQTAAKNVILFLGDGMGVPTVTATRILKGQMNGKLGPETPLAMDQFPYVALSKTYNVDRQVPDSAGTATAYLCGVKGNYKTIGVSAAARYNQCNTTSGNEVTSVMNRAKKAGKSVGVVTTSRVQHASPAGAYAHTVNRNWYSDADLPADAQTYGCQDIATQLVNNMDIDVILGGGRMYMFPEGTPDPEYPYDVNQTGVRKDKRNLVQEWQAKHQGAQYVWNRTELLQAANDPSVTHLMGLFEPADMKYNVQQDPTKDPTLEEMTEAALQVLSRNPQGFYLFVEGGRIDHGHHEGKAYMALTDTVMFDNAIAKANELTSELDTLILATADHSHVFSFGGYTLRGTSIFGLAPSKASDNKSYTSILYGNGPGYVLGGGLRPDVNDSISEDPSYRQQAAVPLSSESHGGEDVAVFARGPQAHLVHGVQEETFVAHVMAFAGCVEPYTDCNLAPPAGTTDAAHPIEGRSVVPALLPLRAGTLLLLETATAP

SEQ ID NO: 12 - DNA, 1669 bp, Artificial Sequence
  Synthetic polymer
atgcaggggccctgggtgctgctgctgctgggcctgaggctacagctctccctgggcgtcatcccaggtaatgaggctccccaagctgttccacacacagggcaccccctcagccaggctgacctgatctctactctccccctggccagctgaggaggagaacccggccttctggaaccgccaggcagctgaggccctggatgctgccaagaagctgcagcccatccagaaggtcgccaagaacctcatcctcttcctgggcgatgggttgggggtgcccacggtgacagccaccaggatcctaaaggggcagaagaatggcaaactggggcctgagacgcccctggccatggaccgcttcccatacctggctctgtccaagacatacaatgtggacagacaggtgccagacagcgcagccacagccacggcctacctgtgcggggtcaaggccaacttccagaccatcggcttgagtgcagccgcccgctttaaccagtgcaacacgacacgcggcaatgaggtcatctccgtgatgaaccgggccaagcaagcaggaaagtcagtaggagtggtgaccaccacacgggtgcagcacgcctcgccagccggcacctacgcacacacagtgaaccgcaactggtactcagatgctgacatgcctgcctcagcccgccaggaggggtgccaggacatcgccactcagctcatctccaacatggacattgacgtgatccttggcggaggccgcaagtacatgtttcccatggggaccccagaccctgagtacccagctgatgccagccagaatggaatcaggctggacgggaagaacctggtgcaggaatggctggcaaagcaccagggtgcctggtatgtgtggaaccgcactgagctcatgcaggcgtccctggaccagtctgtgacccatctcatgggcctctttgagcccggagacacgaaatatgagatccaccgagaccccacactggacccctccctgatggagatgacagaggctgccctgcgcctgctgagcaggaacccccgcggcttctacctctttgtggagggcggccgcatcgaccatggtcatcatgagggtgtggcttaccaggcactcactgaggcggtcatgttcgacgacgccattgagagggcgggccagctcaccagcgaggaggacacgctgaccctcgtcaccgctgaccactcccatgtcttctcctttggtggctacaccttgcgagggagctccatcttcgggttggcccccagcaaggctcaggacagcaaagcctacacgtccatcctgtacggcaatggcccgggctacgtgttcaactcaggcgtgcgaccagacgtgaatgagagcgagagcgggagccccgattaccagcagcaggcggcggtgcccctgtcgtccgagacccacggaggcgaagacgtggcggtgtttgcgcgcggcccgcaggcgcacctggtgcatggtgtgcaggagcagagcttcgtagcgcatgtcatggccttcgctgcctgtctggagccctacacggcctgcgacctggcgcctcccgcctgcaccaccgacgccgcgcacccagttgccgcgtcgctgccactgctggccgggaccctgctgctgctgggggcgtccgctgctccctga

SEQ ID NO: 13 - DNA, 1671 bp, Artificial Sequence
  Synthetic polymer
atgcaggggccctgggtgctgctgctgctgggcctgaggctacagctctccctgggcgtcatcccagctgaggaggagaacccggccttctggaaccgccaggcagctgaggccctggatgctgccaagaagctgcagcccatccagaaggtcgccaagaacctcatcctcttcctgggcgatgggttgggggtgcccacggtgacagccaccaggatcctaaaggggcagaagaatggcaaactggggcctgagacgcccctggccatggaccgcttcccatacctggctctgtccaagacatacaatgtggacagacaggtgccagacagcgcagccacagccacggcctacctgtgcggggtcaaggccaacttccagaccatcggcttgagtgcagccgcccgctttaaccagtgcaacacgacacgcggcaatgaggtcatctccgtgatgaaccgggccaagcaagcaggaaagtcagtaggagtggtgaccaccacacgggtgcagcacgcctcgccagccggcacctacgcacacacagtgaaccgcaactggtactcagatgctgacatgcctgcctcagcccgccaggaggggtgccaggacatcgccactcagctcatctccaacatggacattgacgtgatccttggcggaggccgcaagtacatgtttcccatggggaccccagaccctgagtacccagctgatgccagccagaatggaatcaggctggacgggaagaacctggtgcaggaatggctggcaaagcaccagggtgcctggtatgtgtggaaccgcactgagctcatgcaggcgtccctggaccagtctgtgacccatctcatgggcctctttgagcccggagacacgaaatatgagatccaccgagaccccacactggacccctccctgatggagatgacagaggctgccctgcgcctgctgagcaggaacccccgcggcttctacctctttgtggagggcggccgcatcgaccatggtcatcatgagggtgtggcttaccaggcactcactgaggcggtcatgttcgacgacgccattgagagggcgggccagctcaccagcgaggaggacacgctgaccctcgtcaccgctgaccactcccatgtcttctcctttggtggctacaccttgcgagggagctccatcttcgggttggcccccagcaaggctcaggacagcaaagcctacacgtccatcctgtacggcaatggcccgggctacgtgttcaactcaggcgtgcgaccagacgtgaatgagagcgagagcgggagccccgattaccagcagcaggcggcggtgcccctgtcgtccgagacccacggaggcgaagacgtggcggtgtttgcgcgcggcccgcaggcgcacctggtgcatggtgtgcaggagcagagcttcgtagcgcatgtcatggccttcgctgcctgtctggagccctacacggcctgcgacctggcgcctcccgcctgcaccaccgacgccgcgcacccagttgccgcgtcgctgccactgctggccgggaccctgctgctgctgggggcgtccgctgctccctgatttactaaaaccttgaaataaaattgtaaaacatcagtttgaaggcctgactctcagggtagttcttttttaattctgggtttt

SEQ ID NO: 14 - DNA, 1672 bp, Artificial Sequence
  Synthetic polymer
atgcagtgggcctgtgtgctgctgctgctgggcctgtggctacagctctccctcaccttcatcccaggtaatcaggcggctcccagcagcccctactcacaggggcggctctaggctgacctgaccaacactctccccttgggcagctgaggaggaagaccccgccttctggaaccgccaggcagcccaggcccttgatgtagccaagaagttgcagccgatccagacagctgccaagaatgtcatcctcttcttgggggatgggatgggggtgcctacggtgacagccactcggatcctaaaggggcagatgaatggtaagctgggacctgagacacccctggccatggaccagttcccatacgtggctctgtccaagacatacaacgtggacagacaggtgccagacagcgcaggcactgccactgcctacctgtgtggggtcaagggcaactacaaaaccattggtgtaagtgcagccgcccgctacaaccagtgcaacacaacaagtggcaatgaggtcacgtctgtgatgaaccgggccaagaaagcaggaaagtcagtgggagtggtgaccacctccagggtgcagcatgcctccccagccggtgcttatgcacacacggtgaaccgaaactggtactcagatgccgacctgcctgccgatgcacagacgtatggctgccaggacatcgccacacaactggtcaacaacatggatattgacgtgatcctgggtggaggccgaatgtacatgtttcctgaggggaccccggatcctgaatacccatacgatgtcaatcagactggagtccggaaggacaagcggaatctggtgcaggagtggcaggccaagcaccagggagcccagtatgtgtggaaccgcacggagctccttcaggcagccaatgaccccagtgtaacacacctcatgggcctctttgagccggcagacatgaagtataatgttcagcaagaccccaccaaggacccgaccctggaggagatgacggaggcggccctgcaagtgctgagcaggaacccccagggcttctacctcttcgtggagggaggccgcattgaccacggtcaccatgaaggcaaagcttatatggcactgactgatacagtcatgtttgacaatgccatcgccaaggctaacgagctcactagcgaactggacacgctgatccttgccactgcagaccactcccatgtcttctcttttggtggctacacactgcgtgggacctccattttcggtctggcccccagcaaggcctcagacaacaagtcctacacctccatcctctatggcaatggccctggctacgtgcttggtgggggcttaaggcccgatgttaatgacagcataagcgaggacccctcgtaccggcagcaggcggccgtgcccctgtctagtgagtcccacgggggcgaggacgtggcggtgttcgcgcgaggcccgcaggcgcacctggtgcacggcgtgcaggaggagaccttcgtggcgcacgtcatggcctttgcgggctgcgtggagccctacaccgactgcaatctgccggccccctctggcctctccgacgccgcgcacctggcggccagcccgccttcgctggcgctgctggccggggcgatgctgctgctgctggcgcctgccttgtactga

SEQ ID NO: 15 - DNA, 1869 bp, Artificial Sequence
  Synthetic polymer
atgcagtgggcctgtgtgctgctgctgctgggcctgtggctacagctctccctcaccttcatcccagctgaggaggaagaccccgccttctggaaccgccaggcagcccaggcccttgatgtagccaagaagttgcagccgatccagacagctgccaagaatgtcatcctcttcttgggggatgggatgggggtgcctacggtgacagccactcggatcctaaaggggcagatgaatggtaagctgggacctgagacacccctggccatggaccagttcccatacgtggctctgtccaagacatacaacgtggacagacaggtgccagacagcgcaggcactgccactgcctacctgtgtggggtcaagggcaactacaaaaccattggtgtaagtgcagccgcccgctacaaccagtgcaacacaacaagtggcaatgaggtcacgtctgtgatgaaccgggccaagaaagcaggaaagtcagtgggagtggtgaccacctccagggtgcagcatgcctccccagccggtgcttatgcacacacggtgaaccgaaactggtactcagatgccgacctgcctgccgatgcacagacgtatggctgccaggacatcgccacacaactggtcaacaacatggatattgacgtgatcctgggtggaggccgaatgtacatgtttcctgaggggaccccggatcctgaatacccatacgatgtcaatcagactggagtccggaaggacaagcggaatctggtgcaggagtggcaggccaagcaccagggagcccagtatgtgtggaaccgcacggagctccttcaggcagccaatgaccccagtgtaacacacctcatgggcctctttgagccggcagacatgaagtataatgttcagcaagaccccaccaaggacccgaccctggaggagatgacggaggcggccctgcaagtgctgagcaggaacccccagggcttctacctcttcgtggagggaggccgcattgaccacggtcaccatgaaggcaaagcttatatggcactgactgatacagtcatgtttgacaatgccatcgccaaggctaacgagctcactagcgaactggacacgctgatccttgccactgcagaccactcccatgtcttctcttttggtggctacacactgcgtgggacctccattttcggtctggcccccagcaaggcctcagacaacaagtcctacacctccatcctctatggcaatggccctggctacgtgcttggtgggggcttaaggcccgatgttaatgacagcataagcgaggacccctcgtaccggcagcaggcggccgtgcccctgtctagtgagtcccacgggggcgaggacgtggcggtgttcgcgcgaggcccgcaggcgcacctggtgcacggcgtgcaggaggagaccttcgtggcgcacgtcatggcctttgcgggctgcgtggagccctacaccgactgcaatctgccggccccctctggcctctccgacgccgcgcacctggcggccagcccgccttcgctggcgctgctggccggggcgatgctgctgctgctggcgcctgccttgtactgaggggacccgggggtggggacacaggccccgccctccctgggaggcaggaagcagctctcaaataaactgttctaagtatgatacaggagtgatacatgtgtgaagagaagcccttaggtgggggcacagagtgtctgggtgaggggggtcagggtcacatcaggaggttagggaggggttgatgaagggctgacgttgagcaaagaccaaaggcaactcagaaggacagtggtgcaggactgggtgtggtcagcagggggactggttgggggatcc

SEQ ID NO: 16 - DNA, 1260 bp, Artificial Sequence
  Synthetic polymer
aaaaaacaagacaaagctgagatcagaaatgtcattgtgatgataggcgacggcatggggacgccttacataagagcctaccgttccatgaaaaataacggtgacacaccgaataacccgaagttaacagaatttgaccggaacctgacaggcatgatgatgacgcatccggatgaccctgactataatattacagattcagcagcagccggaacagcattagcgacaggcgttaagacatataacaatgcaattggcgtcgataaaaacggaaaaaaagtgaaatctgtacttgaagaggccaaacagcaaggcaagtcaacagggcttgtcgccacgtctgaaattaaccacgccactccagccgcatatggcgcccacaatgaatcacggaaaaacatggaccaaatcgccaacagctatatggatgacaagataaaaggcaaacataaaatagacgtgctgctcggcggcggaaaatcttattttaaccgcaagaacagaaacttgacaaaggaattcaaacaagccggctacagctatgtgacaactaaacaagcattgaaaaaaaataaagatcagcaggtgctcgggcttttcgcagatggagggcttgctaaagcgctcgaccgtgacagtaaaacaccgtctctcaaagacatgacggtttcagcaattgatcgcctgaaccaaaataaaaaaggatttttcttgatggtcgaagggagccagattgactgggcggcccatgacaatgatacagtaggagccatgagcgaggttaaagattttgaacaggcctataaagccgcgattgaatttgcgaaaaaagacaaacatacacttgtgattgcaactgctgaccatacaaccggcggctttaccattggcgcaaacggggaaaagaattggcacgcagaaccgattctctccgctaagaaaacacctgaattcatggccaaaaaaatcagtgaaggcaagccggttaaagatgtgctcgcccgctatgccaatctgaaagtcacatctgaagaaatcaaaagcgttgaagcagctgcacaggctgacaaaagcaaaggggcctccaaagccatcatcaagatttttaatacccgctccaacagcggatggacgagtaccgatcataccggcgaagaagtaccggtatacgcgtacggccccggaaaagaaaaattccgcggattgattaacaatacggaccaggcaaacatcatatttaagattttaaaaactggaaaa

SEQ ID NO: 17 - protein, 420 aa, Artificial Sequence
  Synthetic polymer
KKQDKAEIRNVIVMIGDGMGTPYIRAYRSMKNNGDTPNNPKLTEFDRNLTGMMMTHPDDPDYNITDSAAAGTALATGVKTYNNAIGVDKNGKKVKSVLEEAKQQGKSTGLVATSEINHATPAAYGAHNESRKNMDQIANSYMDDKIKGKHKIDVLLGGGKSYFNRKNRNLTKEFKQAGYSYVTTKQALKKNKDQQVLGLFADGGLAKALDRDSKTPSLKDMTVSAIDRLNQNKKGFFLMVEGSQIDWAAHDNDTVGAMSEVKDFEQAYKAAIEFAKKDKHTLVIATADHTTGGFTIGANGEKNWHAEPILSAKKTPEFMAKKISEGKPVKDVLARYANLKVTSEEIKSVEAAAQADKSKGASKAIIKIFNTRSNSGWTSTDHTGEEVPVYAYGPGKEKFRGLINNTDQANIIFKILKTGK

SEQ ID NO: 18 - protein, 776 aa, Artificial Sequence
  Synthetic polymer
MQGPWVLLLLGLRLQLSLGVIPAEEENPAFWNRQAAEALDAAKKLQPIQKVAKNLILFLGDGLGVPTVTATRILKGQKNGKLGPETPLAMDRFPYLALSKTYNVDRQVPDSAATATAYLCGVKANFQTIGLSAAARFNQCNTTRGNEVISVMNRAKQAGKSVGVVTTTRVQHASPAGTYAHTVNRNWYSDADMPASARQEGCQDIATQLISNMDIDVILGGGRKYMFPMGTPDPEYPADASQNGIRLDGKNLVQEWLAKHQGAWYVWNRTELMQASLDQSVTHLMGLFEPGDTKYEIHRDPTLDPSLMEMTEAALRLLSRNPRGFYLFVEGGRIDHGHHEGVAYQALTEAVMFDDAIERAGQLTSEEDTLTLVTADHSHVFSFGGYTLRGSSIFGLAPSKAQDSKAYTSILYGNGPGYVFNSGVRPDVNESESGSPDYQQQAAVPLSSETHGGEDVAVFARGPQAHLVHGVQEQSFVAHVMAFAACLEPYTACDLAPPACTTDAAHPVAASLPLLAGTLLLLGASAAPGGSGGSGGGGSGGGGSEPKSCDKTHTCPPCPAPELLGGPSVFLFPPKPKDTLMISRTPEVTCVVVDVSHEDPQVKFNWYVDGVQVHNAKTKPREQQYNSTYRVVSVLTVLHQNWLDGKEYKCKVSNKALPAPIEKTISKAKGQPREPQVYTLPPSREEMTKNQVSLTCLVKGFYPSDIAVEWESNGQPENNYKTTPPVLDSDGSFFLYSKLTVDKSRWQQGNVFSCSVMHEALHNHYTQKSLSLSPGK